European Patent Application EP 4 364 809 A2, published May 8, 2024. Title: CD19 SPECIFIC CHIMERIC ANTIGEN RECEPTOR AND USES THEREOF. Applicant: CELLECTIS. Application EP EP24163057.3, filed May 12, 2014. The sequence listing filed with the application follows.

SEQUENCE LISTING (24 sequences)

SEQ ID NO: 1 - protein, 464 aa, Mus musculus
  REGION 1..464: note = anti-human CD19 monoclonal antibody 4G7 immunoglobulin gamma1 heavy chain
MEWSWIFLFLLSGTAGVHSEVQLQQSGPELIKPGASVKMSCKASGYTFTSYVMHWVKQKPGQGLEWIGYINPYNDGTKYNEKFKGKATLTSDKSSSTAYMELSSLTSEDSAVYYCARGTYYYGSRVFDYWGQGTTLTVSSAKTTPPSVYPLAPGSAAQTNSMVTLGCLVKGYFPEPVTVTWNSGSLSSGVHTFPAVLQSDLYTLSSSVTVPSSTWPSETVTCNVAHPASSTKVDKKIVPRDCGCKPCICTVPEVSSVFIFPPKPKDVLTITLTPKVTCVVVDISKDDPEVQFSWFVDDVEVHTAQTQPREEQFNSTFRSVSELPIMHQDWLNGKEFKCRVNSAAFPAPIEKTISKTKGRPKAPQVYTIPPPKEQMAKDKVSLTCMITDFFPEDITVEWQWNGQPAENYKNTQPIMDTDGSYFVYSKLNVQKSNWEAGNTFTCSVLHEGLHNHHTEKSLSHSPGK

SEQ ID NO: 2 - protein, 239 aa, Mus musculus
  REGION 1..239: note = anti-human CD19 monoclonal antibody 4G7 immunoglobulin kappa light chain
MRCLAEFLGLLVLWIPGAIGDIVMTQAAPSIPVTPGESVSISCRSSKSLLNSNGNTYLYWFLQRPGQSPQLLIYRMSNLASGVPDRFSGSGSGTAFTLRISRVEAEDVGVYYCMQHLEYPFTFGAGTKLELKRADAAPTVSIFPPSSEQLTSGGASVVCFLNNFYPKDINVKWKIDGSERQNGVLNSWTDQDSKDSTYSMSSTLTLTKDEYERHNSYTCEATHKTSTSPIVKSFNRNEC

SEQ ID NO: 3 - protein, 121 aa, Mus musculus
  REGION 1..121: note = fragment of anti-human CD19 monoclonal antibody 4G7 immunoglobulin gamma1 heavy chain-(residues 20-140)
EVQLQQSGPELIKPGASVKMSCKASGYTFTSYVMHWVKQKPGQGLEWIGYINPYNDGTKYNEKFKGKATLTSDKSSSTAYMELSSLTSEDSAVYYCARGTYYYGSRVFDYWGQGTTLTVSS

SEQ ID NO: 4 - protein, 115 aa, Mus musculus
  REGION 1..115: note = fragment of anti-human CD19 monoclonal antibody 4G7 immunoglobulin kappa light chain (residues 21-130)
DIVMTQAAPSIPVTPGESVSISCRSSKSLLNSNGNTYLYWFLQRPGQSPQLLIYRMSNLASGVPDRFSGSGSGTAFTLRISRVEAEDVGVYYCMQHLEYPFTFGAGTKLELKRAD

SEQ ID NO: 5 - protein, 116 aa, synthetic construct
  REGION 1..116: note = fragment of anti-human CD19 monoclonal antibody 4G7 immunoglobulin kappa light chain
DIVMTQAAPSIPVTPGESVSISCRSSKSLLNSNGNTYLYWFLQRPGQSPQLLIYRMSNLASGVPDRFSGSGSGTAFTLRISRVEAEDVGVYYCMQHLEYPFTFGAGTKLELKRSDP

SEQ ID NO: 6 - protein, 15 aa, synthetic construct
  REGION 1..15: note = description of artificial sequence: synthetic oligopeptide
  REGION 1..15: note = Linker
GGGGSGGGGSGGGGS

SEQ ID NO: 7 - protein, 252 aa, synthetic construct
  REGION 1..252: note = description of artificial sequence: synthetic polypeptide
  REGION 1..252: note = scFV 4G7 version 1
EVQLQQSGPELIKPGASVKMSCKASGYTFTSYVMHWVKQKPGQGLEWIGYINPYNDGTKYNEKFKGKATLTSDKSSSTAYMELSSLTSEDSAVYYCARGTYYYGSRVFDYWGQGTTLTVSSGGGGSGGGGSGGGGSDIVMTQAAPSIPVTPGESVSISCRSSKSLLNSNGNTYLYWFLQRPGQSPQLLIYRMSNLASGVPDRFSGSGSGTAFTLRISRVEAEDVGVYYCMQHLEYPFTFGAGTKLELKRSDP

SEQ ID NO: 8 - protein, 251 aa, synthetic construct
  REGION 1..251: note = description of artificial sequence: synthetic polypeptide
  REGION 1..251: note = scFV 4G7 version 2
EVQLQQSGPELIKPGASVKMSCKASGYTFTSYVMHWVKQKPGQGLEWIGYINPYNDGTKYNEKFKGKATLTSDKSSSTAYMELSSLTSEDSAVYYCARGTYYYGSRVFDYWGQGTTLTVSSGGGGSGGGGSGGGGSDIVMTQAAPSIPVTPGESVSISCRSSKSLLNSNGNTYLYWFLQRPGQSPQLLIYRMSNLASGVPDRFSGSGSGTAFTLRISRVEAEDVGVYYCMQHLEYPFTFGAGTKLELKRAD

SEQ ID NO: 9 - protein, 250 aa, synthetic construct
  REGION 1..250: note = description of artificial sequence: synthetic polypeptide
  REGION 1..250: note = scFV FMC63
DIQMTQTTSSLSASLGDRVTISCRASQDISKYLNWYQQKPDGTVKLLIYHTSRLHSGVPSRFSGSGSGTDYSLTISNLEQEDIATYFCQQGNTLPYTFGGGTKLEITKAGGGGSGGGGSGGGGSGGGGSEVKLQESGPGLVAPSQSLSVTCTVSGVSLPDYGVSWIRQPPRKGLEWLGVIWGSETTYYNSALKSRLTIIKDNSKSQVFLKMNSLQTDDTAIYYCAKHYYYGGSYAMDYWGQGTSVTVSSD

SEQ ID NO: 10 - protein, 112 aa, Homo sapiens
  REGION 1..112: note = fragment of T-cell surface glycoprotein CD3 zeta chain
RVKFSRSADAPAYQQGQNQLYNELNLGRREEYDVLDKRRGRDPEMGGKPRRKNPQEGLYNELQKDKMAEAYSEIGMKGERRRGKGHDGLYQGLSTATKDTYDALHMQALPPR

SEQ ID NO: 11 - protein, 42 aa, Homo sapiens
  REGION 1..42: note = Fragment of 4-1BB (residues 214-255)
KRGRKKLLYIFKQPFMRPVQTTQEEDGCSCRFPEEEEGGCEL

SEQ ID NO: 12 - protein, 41 aa, Homo sapiens
  REGION 1..41: note = Fragment of T-cell-specific surface glycoprotein CD28
RSKRSRGGHSDYMNMTPRRPGPTRKHYQPYAPPRDFAAYRS

SEQ ID NO: 13 - protein, 69 aa, Homo sapiens
  REGION 1..69: note = Fragment of T-cell surface glycoprotein CD8 alpha chain isoform 1 precursor (residues 138-206)
TTTPAPRPPTPAPTIASQPLSLRPEACRPAAGGAVHTRGLDFACDIYIWAPLAGTCGVLLLSLVITLYC

SEQ ID NO: 14 - protein, 495 aa, synthetic construct
  REGION 1..495: note = description of artificial sequence: synthetic polypeptide
  REGION 1..495: note = 4G7-CAR version 1
MALPVTALLLPLALLLHAARPEVQLQQSGPELIKPGASVKMSCKASGYTFTSYVMHWVKQKPGQGLEWIGYINPYNDGTKYNEKFKGKATLTSDKSSSTAYMELSSLTSEDSAVYYCARGTYYYGSRVFDYWGQGTTLTVSSGGGGSGGGGSGGGGSDIVMTQAAPSIPVTPGESVSISCRSSKSLLNSNGNTYLYWFLQRPGQSPQLLIYRMSNLASGVPDRFSGSGSGTAFTLRISRVEAEDVGVYYCMQHLEYPFTFGAGTKLELKRADTTTPAPRPPTPAPTIASQPLSLRPEACRPAAGGAVHTRGLDFACDIYIWAPLAGTCGVLLLSLVITLYCKRGRKKLLYIFKQPFMRPVQTTQEEDGCSCRFPEEEEGGCELRVKFSRSADAPAYQQGQNQLYNELNLGRREEYDVLDKRRGRDPEMGGKPRRKNPQEGLYNELQKDKMAEAYSEIGMKGERRRGKGHDGLYQGLSTATKDTYDALHMQALPPR

SEQ ID NO: 15 - protein, 495 aa, synthetic construct
  REGION 1..495: note = description of artificial sequence: synthetic polypeptide
  REGION 1..495: note = 4G7-CAR version 2
METDTLLLWVLLLWVPGSTGEVQLQQSGPELIKPGASVKMSCKASGYTFTSYVMHWVKQKPGQGLEWIGYINPYNDGTKYNEKFKGKATLTSDKSSSTAYMELSSLTSEDSAVYYCARGTYYYGSRVFDYWGQGTTLTVSSGGGGSGGGGSGGGGSDIVMTQAAPSIPVTPGESVSISCRSSKSLLNSNGNTYLYWFLQRPGQSPQLLIYRMSNLASGVPDRFSGSGSGTAFTLRISRVEAEDVGVYYCMQHLEYPFTFGAGTKLELKRSDPTTTPAPRPPTPAPTIASQPLSLRPEACRPAAGGAVHTRGLDFACDIYIWAPLAGTCGVLLLSLVITLYCKRGRKKLLYIFKQPFMRPVQTTQEEDGCSCRFPEEEEGGCELRVKFSRSADAPAYQQGQNQLYNELNLGRREEYDVLDKRRGRDPEMGGKPRRKNPQEGLYNELQKDKMAEAYSEIGMKGERRRGKGHDGLYQGLSTATKDTYDALHMQALPPR

SEQ ID NO: 16 - protein, 494 aa, synthetic construct
  REGION 1..494: note = description of artificial sequence: synthetic polypeptide
  REGION 1..494: note = FMC63-CAR
METDTLLLWVLLLWVPGSTGDIQMTQTTSSLSASLGDRVTISCRASQDISKYLNWYQQKPDGTVKLLIYHTSRLHSGVPSRFSGSGSGTDYSLTISNLEQEDIATYFCQQGNTLPYTFGGGTKLEITKAGGGGSGGGGSGGGGSGGGGSEVKLQESGPGLVAPSQSLSVTCTVSGVSLPDYGVSWIRQPPRKGLEWLGVIWGSETTYYNSALKSRLTIIKDNSKSQVFLKMNSLQTDDTAIYYCAKHYYYGGSYAMDYWGQGTSVTVSSDPTTTPAPRPPTPAPTIASQPLSLRPEACRPAAGGAVHTRGLDFACDIYIWAPLAGTCGVLLLSLVITLYCKRGRKKLLYIFKQPFMRPVQTTQEEDGCSCRFPEEEEGGCELRVKFSRSADAPAYQQGQNQLYNELNLGRREEYDVLDKRRGRDPEMGGKPRRKNPQEGLYNELQKDKMAEAYSEIGMKGERRRGKGHDGLYQGLSTATKDTYDALHMQALPPR

SEQ ID NO: 17 - DNA, 1488 bp, synthetic construct
  misc_feature 1..1488: note = description of artificial sequence: synthetic polynucleotide
  misc_feature 1..1488: note = 4G7-CAR version 2
  source 1..1488: mol_type = other DNA
atggagaccgacaccctgctgctgtgggtgctgctgctgtgggtgccaggcagcaccggcgaggtgcagctgcagcagagcggacccgagctgatcaagccaggcgccagcgtgaagatgagctgcaaggccagcggctacaccttcaccagctacgtgatgcactgggtgaagcagaagccaggccagggcctggagtggatcggctacatcaacccctacaacgacggcaccaagtacaacgagaagttcaagggcaaggccaccctgaccagcgacaagagcagcagcaccgcctacatggagctgagcagcctgaccagcgaggacagcgccgtgtactactgcgccagaggcacctactactacggcagccgggtgttcgactactggggccagggcaccaccctgaccgtgagctctggcggaggcggctctggcggaggcggctctggcggaggcggcagcgacatcgtgatgacccaggctgcccccagcatccccgtgaccccaggcgagagcgtgagcatcagctgccggagcagcaagagcctgctgaacagcaacggcaacacctacctgtactggttcctgcagcggccaggccagagcccccagctgctgatctaccggatgagcaacctggccagcggcgtgcccgaccggttcagcggcagcggcagcggcaccgccttcaccctgcggatcagccgggtggaggccgaggacgtgggcgtgtactactgcatgcagcacctggagtaccccttcaccttcggagccggcaccaagctggagctgaagcggtcggatcccaccaccaccccagccccacggccacctacccctgccccaaccatcgccagccagcccctgagcctgcggcctgaagcctgcaggcctgccgccggaggagccgtgcacacaaggggcctggacttcgcctgcgacatctatatctgggcccccctggccgggacatgcggggtgctgctgctgtccctggtgattacactgtattgcaaacggggccggaagaagctgctgtacatcttcaagcagcccttcatgcggcccgtgcagaccacccaggaggaggacggctgcagctgccggttccccgaggaagaggaaggcggctgcgagctgcgggtgaagttcagccggagcgccgacgccccagcctaccagcagggccagaaccagctgtacaacgagctgaacctgggacggcgggaggagtacgacgtgctggacaagcggcggggacgggaccccgagatgggcggcaagcctcgccggaagaatccccaggagggcctgtacaacgagctgcagaaggacaagatggccgaggcctacagcgagatcggcatgaagggcgagcggcgccggggcaagggccacgacggcctgtaccagggcctgagcaccgccaccaaggacacctacgacgccctgcacatgcaggccctgccaccccggtga

SEQ ID NO: 18 - protein, 20 aa, synthetic construct
  REGION 1..20: note = description of artificial sequence: synthetic oligopeptide
  REGION 1..20: note = signal peptide
METDTLLLWVLLLWVPGSTG

SEQ ID NO: 19 - protein, 21 aa, synthetic construct
  REGION 1..21: note = description of artificial sequence: synthetic oligopeptide
  REGION 1..21: note = signal peptide
MALPVTALLLPLALLLHAARP

SEQ ID NO: 20 - DNA, 49 bp, synthetic construct
  source 1..49: mol_type = other DNA
  misc_feature 1..49: note = Description of Artificial Sequence: Synthetic oligonucleotide
ttgtcccacagatatccagaaccctgaccctgccgtgtaccagctgaga

SEQ ID NO: 21 - protein, 530 aa, synthetic construct
  REGION 1..530: note = Description of Artificial Sequence: Synthetic polypeptide
  REGION 1..530: note = Repeat TRAC_T01-L
LTPQQVVAIASNGGGKQALETVQRLLPVLCQAHGLTPQQVVAIASNNGGKQALETVQRLLPVLCQAHGLTPQQVVAIASNGGGKQALETVQRLLPVLCQAHGLTPEQVVAIASHDGGKQALETVQRLLPVLCQAHGLTPEQVVAIASHDGGKQALETVQRLLPVLCQAHGLTPEQVVAIASHDGGKQALETVQRLLPVLCQAHGLTPEQVVAIASNIGGKQALETVQALLPVLCQAHGLTPEQVVAIASHDGGKQALETVQRLLPVLCQAHGLTPEQVVAIASNIGGKQALETVQALLPVLCQAHGLTPQQVVAIASNNGGKQALETVQRLLPVLCQAHGLTPEQVVAIASNIGGKQALETVQALLPVLCQAHGLTPQQVVAIASNGGGKQALETVQRLLPVLCQAHGLTPEQVVAIASNIGGKQALETVQALLPVLCQAHGLTPQQVVAIASNGGGKQALETVQRLLPVLCQAHGLTPEQVVAIASHDGGKQALETVQRLLPVLCQAHGLTPQQVVAIASNGGGRPALE

SEQ ID NO: 22 - protein, 530 aa, synthetic construct
  REGION 1..530: note = Description of Artificial Sequence: Synthetic polypeptide
  REGION 1..530: note = Repeat TRAC_T01-R
LTPEQVVAIASHDGGKQALETVQRLLPVLCQAHGLTPQQVVAIASNGGGKQALETVQRLLPVLCQAHGLTPEQVVAIASHDGGKQALETVQRLLPVLCQAHGLTPEQVVAIASNIGGKQALETVQALLPVLCQAHGLTPQQVVAIASNNGGKQALETVQRLLPVLCQAHGLTPEQVVAIASHDGGKQALETVQRLLPVLCQAHGLTPQQVVAIASNGGGKQALETVQRLLPVLCQAHGLTPQQVVAIASNNGGKQALETVQRLLPVLCQAHGLTPQQVVAIASNNGGKQALETVQRLLPVLCQAHGLTPQQVVAIASNGGGKQALETVQRLLPVLCQAHGLTPEQVVAIASNIGGKQALETVQALLPVLCQAHGLTPEQVVAIASHDGGKQALETVQRLLPVLCQAHGLTPEQVVAIASNIGGKQALETVQALLPVLCQAHGLTPEQVVAIASHDGGKQALETVQRLLPVLCQAHGLTPQQVVAIASNNGGKQALETVQRLLPVLCQAHGLTPQQVVAIASNGGGRPALE

SEQ ID NO: 23 - DNA, 2814 bp, synthetic construct
  misc_feature 1..2814: note = Description of Artificial Sequence: Synthetic polynucleotide
  misc_feature 1..2814: note = TRAC_T01-R TALEN
  source 1..2814: mol_type = other DNA
atgggcgatcctaaaaagaaacgtaaggtcatcgattacccatacgatgttccagattacgctatcgatatcgccgatctacgcacgctcggctacagccagcagcaacaggagaagatcaaaccgaaggttcgttcgacagtggcgcagcaccacgaggcactggtcggccacgggtttacacacgcgcacatcgttgcgttaagccaacacccggcagcgttagggaccgtcgctgtcaagtatcaggacatgatcgcagcgttgccagaggcgacacacgaagcgatcgttggcgtcggcaaacagtggtccggcgcacgcgctctggaggccttgctcacggtggcgggagagttgagaggtccaccgttacagttggacacaggccaacttctcaagattgcaaaacgtggcggcgtgaccgcagtggaggcagtgcatgcatggcgcaatgcactgacgggtgccccgctcaacttgaccccccagcaggtggtggccatcgccagcaatggcggtggcaagcaggcgctggagacggtccagcggctgttgccggtgctgtgccaggcccacggcttgaccccccagcaggtggtggccatcgccagcaataatggtggcaagcaggcgctggagacggtccagcggctgttgccggtgctgtgccaggcccacggcttgaccccccagcaggtggtggccatcgccagcaatggcggtggcaagcaggcgctggagacggtccagcggctgttgccggtgctgtgccaggcccacggcttgaccccggagcaggtggtggccatcgccagccacgatggcggcaagcaggcgctggagacggtccagcggctgttgccggtgctgtgccaggcccacggcttgaccccggagcaggtggtggccatcgccagccacgatggcggcaagcaggcgctggagacggtccagcggctgttgccggtgctgtgccaggcccacggcttgaccccggagcaggtggtggccatcgccagccacgatggcggcaagcaggcgctggagacggtccagcggctgttgccggtgctgtgccaggcccacggcttgaccccggagcaggtggtggccatcgccagcaatattggtggcaagcaggcgctggagacggtgcaggcgctgttgccggtgctgtgccaggcccacggcttgaccccggagcaggtggtggccatcgccagccacgatggcggcaagcaggcgctggagacggtccagcggctgttgccggtgctgtgccaggcccacggcttgaccccggagcaggtggtggccatcgccagcaatattggtggcaagcaggcgctggagacggtgcaggcgctgttgccggtgctgtgccaggcccacggcttgaccccccagcaggtggtggccatcgccagcaataatggtggcaagcaggcgctggagacggtccagcggctgttgccggtgctgtgccaggcccacggcttgaccccggagcaggtggtggccatcgccagcaatattggtggcaagcaggcgctggagacggtgcaggcgctgttgccggtgctgtgccaggcccacggcttgaccccccagcaggtggtggccatcgccagcaatggcggtggcaagcaggcgctggagacggtccagcggctgttgccggtgctgtgccaggcccacggcttgaccccggagcaggtggtggccatcgccagcaatattggtggcaagcaggcgctggagacggtgcaggcgctgttgccggtgctgtgccaggcccacggcttgaccccccagcaggtggtggccatcgccagcaatggcggtggcaagcaggcgctggagacggtccagcggctgttgccggtgctgtgccaggcccacggcttgaccccggagcaggtggtggccatcgccagccacgatggcggcaagcaggcgctggagacggtccagcggctgttgccggtgctgtgccaggcccacggcttgacccctcagcaggtggtggccatcgccagcaatggcggcggcaggccggcgctggagagcattgttgcccagttatctcgccctgatccggcgttggccgcgttgaccaacgaccacctcgtcgccttggcctgcctcggcgggcgtcctgcgctggatgcagtgaaaaagggattgggggatcctatcagccgttcccagctggtgaagtccgagctggaggagaagaaatccgagttgaggcacaagctgaagtacgtgccccacgagtacatcgagctgatcgagatcgcccggaacagcacccaggaccgtatcctggagatgaaggtgatggagttcttcatgaaggtgtacggctacaggggcaagcacctgggcggctccaggaagcccgacggcgccatctacaccgtgggctcccccatcgactacggcgtgatcgtggacaccaaggcctactccggcggctacaacctgcccatcggccaggccgacgaaatgcagaggtacgtggaggagaaccagaccaggaacaagcacatcaaccccaacgagtggtggaaggtgtacccctccagcgtgaccgagttcaagttcctgttcgtgtccggccacttcaagggcaactacaaggcccagctgaccaggctgaaccacatcaccaactgcaacggcgccgtgctgtccgtggaggagctcctgatcggcggcgagatgatcaaggccggcaccctgaccctggaggaggtgaggaggaagttcaacaacggcgagatcaacttcgcggccgactgataa

SEQ ID NO: 24 - DNA, 2832 bp, synthetic construct
  misc_feature 1..2832: note = Description of Artificial Sequence: Synthetic polynucleotide
  source 1..2832: mol_type = other DNA
atgggcgatcctaaaaagaaacgtaaggtcatcgataaggagaccgccgctgccaagttcgagagacagcacatggacagcatcgatatcgccgatctacgcacgctcggctacagccagcagcaacaggagaagatcaaaccgaaggttcgttcgacagtggcgcagcaccacgaggcactggtcggccacgggtttacacacgcgcacatcgttgcgttaagccaacacccggcagcgttagggaccgtcgctgtcaagtatcaggacatgatcgcagcgttgccagaggcgacacacgaagcgatcgttggcgtcggcaaacagtggtccggcgcacgcgctctggaggccttgctcacggtggcgggagagttgagaggtccaccgttacagttggacacaggccaacttctcaagattgcaaaacgtggcggcgtgaccgcagtggaggcagtgcatgcatggcgcaatgcactgacgggtgccccgctcaacttgaccccggagcaggtggtggccatcgccagccacgatggcggcaagcaggcgctggagacggtccagcggctgttgccggtgctgtgccaggcccacggcttgaccccccagcaggtggtggccatcgccagcaatggcggtggcaagcaggcgctggagacggtccagcggctgttgccggtgctgtgccaggcccacggcttgaccccggagcaggtggtggccatcgccagccacgatggcggcaagcaggcgctggagacggtccagcggctgttgccggtgctgtgccaggcccacggcttgaccccggagcaggtggtggccatcgccagcaatattggtggcaagcaggcgctggagacggtgcaggcgctgttgccggtgctgtgccaggcccacggcttgaccccccagcaggtggtggccatcgccagcaataatggtggcaagcaggcgctggagacggtccagcggctgttgccggtgctgtgccaggcccacggcttgaccccggagcaggtggtggccatcgccagccacgatggcggcaagcaggcgctggagacggtccagcggctgttgccggtgctgtgccaggcccacggcttgaccccccagcaggtggtggccatcgccagcaatggcggtggcaagcaggcgctggagacggtccagcggctgttgccggtgctgtgccaggcccacggcttgaccccccagcaggtggtggccatcgccagcaataatggtggcaagcaggcgctggagacggtccagcggctgttgccggtgctgtgccaggcccacggcttgaccccccagcaggtggtggccatcgccagcaataatggtggcaagcaggcgctggagacggtccagcggctgttgccggtgctgtgccaggcccacggcttgaccccccagcaggtggtggccatcgccagcaatggcggtggcaagcaggcgctggagacggtccagcggctgttgccggtgctgtgccaggcccacggcttgaccccggagcaggtggtggccatcgccagcaatattggtggcaagcaggcgctggagacggtgcaggcgctgttgccggtgctgtgccaggcccacggcttgaccccggagcaggtggtggccatcgccagccacgatggcggcaagcaggcgctggagacggtccagcggctgttgccggtgctgtgccaggcccacggcttgaccccggagcaggtggtggccatcgccagcaatattggtggcaagcaggcgctggagacggtgcaggcgctgttgccggtgctgtgccaggcccacggcttgaccccggagcaggtggtggccatcgccagccacgatggcggcaagcaggcgctggagacggtccagcggctgttgccggtgctgtgccaggcccacggcttgaccccccagcaggtggtggccatcgccagcaataatggtggcaagcaggcgctggagacggtccagcggctgttgccggtgctgtgccaggcccacggcttgacccctcagcaggtggtggccatcgccagcaatggcggcggcaggccggcgctggagagcattgttgcccagttatctcgccctgatccggcgttggccgcgttgaccaacgaccacctcgtcgccttggcctgcctcggcgggcgtcctgcgctggatgcagtgaaaaagggattgggggatcctatcagccgttcccagctggtgaagtccgagctggaggagaagaaatccgagttgaggcacaagctgaagtacgtgccccacgagtacatcgagctgatcgagatcgcccggaacagcacccaggaccgtatcctggagatgaaggtgatggagttcttcatgaaggtgtacggctacaggggcaagcacctgggcggctccaggaagcccgacggcgccatctacaccgtgggctcccccatcgactacggcgtgatcgtggacaccaaggcctactccggcggctacaacctgcccatcggccaggccgacgaaatgcagaggtacgtggaggagaaccagaccaggaacaagcacatcaaccccaacgagtggtggaaggtgtacccctccagcgtgaccgagttcaagttcctgttcgtgtccggccacttcaagggcaactacaaggcccagctgaccaggctgaaccacatcaccaactgcaacggcgccgtgctgtccgtggaggagctcctgatcggcggcgagatgatcaaggccggcaccctgaccctggaggaggtgaggaggaagttcaacaacggcgagatcaacttcgcggccgactgataa